European Patent Specification EP 3 434 276 B1, published October 30, 2024. Title: METHOD AND PHARMACEUTICAL COMPOSITION FOR USE IN THE TREATMENT OF CANCER. Applicant: INSERM. The sequence listing filed with the application follows.

SEQUENCE LISTING (5 sequences)

SEQ ID NO: 1 - protein, 10 aa, Artificial
  peptide
KRFYVVMWKK

SEQ ID NO: 2 - protein, 10 aa, Artificial
  Peptide
KRFYGGMWKK

SEQ ID NO: 3 - protein, 8 aa, Artificial
  peptide
RFYVVMWK

SEQ ID NO: 4 - protein, 8 aa, Artificial
  peptide
KWMVVYFR

SEQ ID NO: 5 - protein, 10 aa, Artificial
  peptide
KKWMVVYFRK